European Patent Specification EP 3 489 680 B1, published July 3, 2024. Title: METHOD OF DETERMINING ACUTE MYELOID LEUKEMIA RESPONSE TO TREATMENT WITH FARNESYLTRANSFERASE INHIBITORS. Applicant: Janssen Diagnostics, LLC. The sequence listing filed with the application follows.

SEQUENCE LISTING (12 sequences)

SEQ ID NO: 1 - DNA, 79 bp, Artificial Sequence
  RASGRP1 Amplicon
ctggacgatctcattgacagctgcattcaatcttttgatgcagatggaaacctgtgtcgaagtaaccaactgttgcaag

SEQ ID NO: 2 - DNA, 78 bp, Artificial Sequence
  APTX Amplicon
cgcttccgattgggctaccacgccattccgagtatgagccatgtacatcttcatgtgatcagccaggattttgattct

SEQ ID NO: 3 - DNA, 18 bp, Artificial Sequence
  APTX upper primer
cgcttccgattgggctac

SEQ ID NO: 4 - DNA, 22 bp, Artificial Sequence
  APTX lower primer
agaatcaaaatcctggctgatc

SEQ ID NO: 5 - DNA, 21 bp, Artificial Sequence
  RASGPR1 upper primer
ctggacgatctcattgacagc

SEQ ID NO: 6 - DNA, 22 bp, Artificial Sequence
  RASGPR1 lower primer
cttgcaacagttggttacttcg

SEQ ID NO: 7 - DNA, 67 bp, Artificial Sequence
  HMBS Amplicon
cctgcccactgtgcttcctcctggcttcaccatcggagccatctgcaagcgggaaaaccctcatgat

SEQ ID NO: 8 - DNA, 19 bp, Artificial Sequence
  HMBS upper primer
cctgcccactgtgcttcct

SEQ ID NO: 9 - DNA, 20 bp, Artificial Sequence
  HMBS lower primer
atcatgagggttttcccgct

SEQ ID NO: 10 - DNA, 31 bp, Artificial Sequence
  RASGPR1 Taqman probe
cattcaatcttttgatgcagatggaaacctg

SEQ ID NO: 11 - DNA, 28 bp, Artificial Sequence
  APTX TaqMan probe
cacgccattccgagtatgagccatgtac

SEQ ID NO: 12 - DNA, 24 bp, Artificial Sequence
  HMBS TaqMan probe
gcttcaccatcggagccatctgca